European Patent Application EP 4 361 281 A2, published May 1, 2024. Title: ACIDOPHILIC FUSARIUM OXYSPORUM STRAINS, METHODS OF THEIR PRODUCTION AND METHODS OF THEIR USE. Applicant: The Fynder Group, Inc. The sequence listing filed with the application follows.

SEQUENCE LISTING (1 sequence)

SEQ ID NO: 1 - DNA, 962 bp, Fusarium oxysporum
  source 1..962: mol_type = genomic DNA; strain = strain MK7
ccgcggggaatactacctgatccgaggtcacattcagagttgggggtttacggcttggccgcgccgcgtaccagttgcgagggttttactactacgcaatggaagctgcagcgagaccgccactagatttcggggccggcttgccgcaagggctcgccgatccccaacaccaaacccgggggcttgagggttgaaatgacgctcgaacaggcatgcccgccagaatactggcgggcgcaatgtgcgttcaaagattcgatgattcactgaattctgcaattcacattacttatcgcattttgctgcgttcttcatcgatgccagaaccaagagatccgttgttgaaagttttgatttatttatggttttactcagaagttacatatagaaacagagtttaggggtcctctggcgggccgtcccgttttaccgggagcgggctgatccgccgaggcaacaattggtatgttcacaggggtttgggagttgtaaactcggtaatgatccctccgcagttctcacctacggataggatcattaccgagtttacaactcccaaacccctgtgaacatacccattgttgcctcggccggatcagcccgctcccggttaaaacgggacggcccgccagagtacccctaaactctgtttctatatgtaacttctgagtaaaaccataaataaatcaaaactttcaacacgcatctcttgcttctgtcatcgatgaagaacgcagcaaaatgcgatagtcatgtgattgcacattcagtgaatcatcgatcttgacgcacattgcgcctgcagtattctggcggtcatgcctgttcgagcgtcattcagccctcagccctcggttgtgttcgggatcggcgagtcctgcgccagcgaccggatcagtggcgtctgcctgcgcctccattgcggttagagttaagccctcgcccacttgttttacgctaac